European Patent Application EP 4 116 419 A1, published January 11, 2023. Title: CALM2 antisense oligonucleotide. Applicant: NISSAN CHEMICAL CORPORATION Kyoto University. Application PCT/JP2021/008514. The sequence listing filed with the application follows.

SEQUENCE LISTING (73 sequences)

SEQ ID NO: 1 - DNA, 1331 bp, Homo sapiens
gaggggagggggttggccgggactcgtttgcgatgttccgttatctggatgcggcggagggatctggcggagggaggtgtttatgaggcgctgggggcggaggaggcgaattagtccgagtggagagagcgagctgagtggttgtgtggtcgcgtctcggaaaccggtagcgcttgcagcatggctgaccaactgactgaagagcagattgcagaattcaaagaagctttttcactatttgacaaagatggtgatggaactataacaacaaaggaattgggaactgtaatgagatctcttgggcagaatcccacagaagcagagttacaggacatgattaatgaagtagatgctgatggtaatggcacaattgacttccctgaatttctgacaatgatggcaagaaaaatgaaagacacagacagtgaagaagaaattagagaagcattccgtgtgtttgataaggatggcaatggctatattagtgctgcagaacttcgccatgtgatgacaaaccttggagagaagttaacagatgaagaagttgatgaaatgatcagggaagcagatattgatggtgatggtcaagtaaactatgaagagtttgtacaaatgatgacagcaaagtgaagaccttgtacagaatgtgttaaatttcttgtacaaaattgtttatttgccttttctttgtttgtaacttatctgtaaaaggtttctccctactgtcaaaaaaatatgcatgtatagtaattaggacttcattcctccatgttttcttcccttatcttactgtcattgtcctaaaaccttattttagaaaattgatcaagtaacatgttgcatgtggcttactctggatatatctaagcccttctgcacatctaaacttagatggagttggtcaaatgagggaacatctgggttatgccttttttaaagtagttttctttaggaactgtcagcatgttgttgttgaagtgtggagttgtaactctgcgtggactatggacagtcaacaatatgtacttaaaagttgcactattgcaaaacgggtgtattatccaggtactcgtacactatttttttgtactgctggtcctgtaccagaaacattttcttttattgttacttgctttttaaactttgtttagccacttaaaatctgcttatggcacaatttgcctcaaaatccattccaagttgtatatttgttttccaataaaaaaattacaatttacccaatggttgctctgcatctgagtcatttaactgttgaagtctaataattttgaaaataaaatatggcattggtttctgcttggtaaaaaaaa

SEQ ID NO: 2 - DNA, 16542 bp, Homo sapiens
gaggggagggggttggccgggactcgtttgcgatgttccgttatctggatgcggcggagggatctggcggagggaggtgtttatgaggcgctgggggcggaggaggcgaattagtccgagtggagagagcgagctgagtggttgtgtggtcgcgtctcggaaaccggtagcgcttgcagcatggtgagtgcatcgctgagctgccggcgctgggcctgtggggggaagagactggagcgaactgactaaacaaaggaaactcgcctcccttacaccttcaaggagtggtttctgccagagggatggcgcgaaagaggccagggatgccggcgacggttgtgtcgcaggtgctcccccacccccattctcttcaggggggcttcctctagtgagttgagggccggacgcacagttcccgaggtggtgaagctcctcgggggcttggctggaggaggatgggtccgggatgagggacagcccagtgcacgggaaggagagaaagtgaaggaagggagagagggagcgtagagagccttctgtcgggcgtctggaaaggtcaagcagggggcgaattcaatccacccgaccgacggttagtgcgggcgccaggaagcgcctttgtccgcttgcggccgccatgcgcccagggggcgggaggagcgcgcggggccctggggcgagcgtcggcgtcgcagttagcccgcgtcctccgcgtgccgggatccagggggcgcgcgggcgggcgggcggcgcgctgtgtgggccgagcccgcgcggcgcagggagcggccggtgggggcggggcgggcgagcgcctcgcgggacccggagccgccgccccgctcggccccgctcgagctccagctgctctgctggcacctgcaggactgcggagatctccttggcgctgcggggccattggcggggatgggcgggggaggggggcctcgacggtttcccatccccctctggcaaccctaatcttccttctccatctgggccctggggcgtcttccaccacccaggccggatgctttaaaaaaaattgctttttaaagtgtctgtcgttgaaagaaattagtcttacccttgaagtcaggggcgcgtcctcgcaatacacatcttgttagggaaagtgttcggctccagctagggttctacaaggcgtttcttgttcaccgccggagggaagcaggctccggagtgactgccttctgaaagtcggtcttgtaacaattggatggatgcctttgaagagcccctgtccctattctatgcttgaaaacagcgtgcagtcctaatgttcaagaaccacgaccacataaaaacattgctccccttctgctgctttgaaaacgacccctaaattccgtgtagaagttgccaggtcgtcttgacgtacacttcgtttgtatgatgtttgtctgtcaaatactgtgatggaagagtgtatgcgggggaggagcagggaatttttaaaagcattttccggtcacctcagactgggagatcatgttctttcctgaaaaaaaaaaaaaaaaacacctaatgagggcggtgatctgtgatacttactttgtggttcctcctgccaagtggttacagcgatgggtgtgtccaggaggcaaggtgacatcttaaacaggagttagggatccttgccaactgaaacctccagcctgtatgggtgtggggagacgatttcaccttaaataaaactagcgttcattgacgtttgatggatttgcttcatcttgatgcttcaaatgttattctgaatttgaatgtgctggttacatttgctttcttaaagatgtagttacaggcatatgtaataaacattacaagttgtggagtaagcttttttttttaaataaacgaagggtaaagttttctttaatcagttttgataattgaatcagtaattcgaatagattttttcttggtagagttggtatctacgcatttgtggtcccttgcccagtgttaagcttttgtagttactgtttgcatcactggtgctttgggggttttctgttaaattgacagctcttactataagagacaaagtcgaaaaaaaaaatcttaataaaaattgacagatatcattatttgtgacagatacagtaaatttgaaaattgccttcacataactttataattagaggactgagattttacattaggaatccaattaaaaaaaattagccggacataatggcctgtgcgtgtagtcctggctagtcaatgggctgaggcaggaggatcatcttgggcccgggagttggagactgtagtgagctatgatcacaccactgcactccctgggcaacagagtgagaccctgtctctcaaaaaataaaaaaaattaggaccccaagttaaagtataaaaaattttatacggaagtaaagtaagattgctcatgtaactcttgagtttacatgtaatcaacatatgctcattgaaaacgggattgcttcaagaggactttgagtgcagggtgattaggtaagtaaaagatgtaaaaaggtagaaaatttttgtcacttgagtctaaataattgttcttataagtgccaacgcctgtttctgttaggctcagaagatcaaaggatttggctcttttaaaatatagaaagctctagcttcagctagaatttaggcctttagtaatagccctaatttttatgaagccattttgttccagtgatcttttggtgagagatgctatgtaagtactattcttcagaattaggtgtctttttaccctaatgaaataatttagattgcttttgatacaggtaaaacaaatatcctggcttccataattgtagaaaaaacttcatataggaatccttgttgtatcaaagtagcacctgatgggaatgaacagacaggaatggatgaaggatagcagtttgcgttccatttcaagcctatgggctcacacatttattcagataagaacaccacctttcactagataaactccaacagtattcatgcatacttttgaatggcatgtaggaaatgtttgataggtacataatgtattcacttcaggtcactaatgtaatacggggtcgtgctccttagtgttgacagatcacctatggttctccaaaatgaacattctagtacaggaggtctagggaggaacctgagagtatactaatgcctaggaactttctctggagtggcaagagcagtgggaagaattatgtcaatagctacagaaataagggagtaagaacaagtcatctctctagtgaattcttcttcactttactgagataaacatacatgttaatgagcttgagttttcccaaaagtataattcttctggttcttctaagaaaatggcactccctggaaacaaggaagaaccaaatttattcgcctttgtagcagttgggaaagttagtgctaggaagtcttcttgatttatagtaggctttaatctggatattgctggtaaaagtttattctaaaacctgaactctggataagtaatacaaaaagcttctcaaccttccaagcaaaattgagagctttcaggttatgtgagtaatttggtctcttgggtgcttaattcattccttgaagctcatttttgtgatctcttccaagattgcatttgcttggaggtagggagttagacaagatggtatgaggtccctaaattttgactttccaagcaaaattggacagtggttcctaaattgctaacatcctcgtttcttcctaaggcttctcatgtttcatatatagtagccttcccaaagtcccatttcccaccccccccccccccccaacccatgtagagagaacgaacctgtctcccttcctgtacagagtacgggatccttcaactttcacacaggctgcagtgtctgccacacatttagctcaacttttttttagccttaaagtgatgtccgctgcatctgtcgctgggttgcaccttgtggatttagtttgcataaattttctcagcttaaacaaagttaacattgaatagagtaagcttaccataaagggcttaataaatgccatgcatgtctacattcggtgtggaaattgagctagtcaggttgatatttaacattgtaggttctttgttaatttatatgaaataatggttatcatttaactctttaggttagctttgtacatagcatctcactttgcacaacaaccctgcaaggtaagtattgttattcttgtgctacaaatgaagttgactgagaggaggagtaccacgtccaaggtcacacagctattaaatggcagggctgggatactggcctgtgactcagaacttgatgctttccccccacgccacgcatgccaggttgcccttcctttcagaaatggtggaagtcctgcaaaatgcaataaactgaagtaatgtagcttctattaatacaaagtaaataactcagatttactggattttaaaccttattccttgggtaaacaatctgtgactgacttcacaccaaatatttgttggcggaggatttggactttagggataaaagtggatacattttttattttacaaactctgtatttgaacttaattattggctcttcaattttacgttaccagcttttttttttttttttttttttaatgaatttgatttacatcatggtcaaacaaaaattgttgagcagggaaaataaactgctttctggattccttcttgaattttctcatgtgccctagagaaaatgtgttccacattaaggtgttactttttccaggggtgtgttcatttaaaaagaatgaagccaggcaatgtttatttttcttttacctataaataaatgaatggattaatcattgtatacttgactcccatgttggtagggattttagataggaggctatttcttgtctgtgcttctcaataccccataagcagttgcttcatggatgtatatactaataagcagtgaaagaaagtgcatgttcaaagaatacaacaaggagtctggatattttgcaatcatctttatatattacggtgctctgaattaaaagctaaaagttactgggtatgtctgacaccttagtgctttatctttgttctactaattttctgtgccccaatcccacttaaccctagcctcattccttatctgtaagataggggataataccactgtaaggttattattaagattgaataaggataaaatttataatgggttttagcaaatggcagaaaatattttctgaagaaaaccaagtgctattaaaaaaacatcacaagccttgggcttactttgggattttaaaaaccaagagaaaatggatggctgaactttcaaacatttggtaaatattatagtactgtagttcagagctctggattctttgcattttgcctgctgggtgagaaggaataaaagtttgtgcctttttttttttttaatcactttaatttcaaaacaatgtgtttaaccatttgtgggagtaattttcattttgtgagcctgaagcattttgattcagtgggaatttctggtgatttatatctggaatagaagtgagcttaagtttagctattctaacgttgaaaaaggaagcaatgtttctattggattctaaagtatattttcaaaaatattctgaagtatttgtatatcttaaacttggagttaagacagcttagctttgaagataagagaaactagatgtgtgcattttctatccagatgtgtttgttgctggaactaaatgaaacagtacatggtaacccttgaaaggttttaaacttgtttctgtaactgctaatctacatactctcaagtcactaaccttcctctttgatctctttgtaggctgaccaactgactgaagagcagattgcaggtgagaaatactcagctagattgtacccattagattcttattataaattgaatagccaacgtcagaataagagacttgtatgaaataattgactttggtatatgtcatggatactaacatatgggtataatataatacagtaattcaacctgctttggcaagtgggattgtaaacttgccgatggaagatgtgcagggctaattgtagttaaagacatgtattttagtctgcgtggatatactttggagccttgtggtgtagtggtggtctttgttttgttttctgaagactaccttagtataaaacaggaattctgggctagctaacacgctagaaaaggaggccaagaagtaactaaggcaacttgaaatggagaatcaaaaaaggaacaattgaatttaccctagttaaaattagctaacattttaacctaagaattgcatatataatcagtcagggaataaccatttctcaagtgaaaaaatttaagaagttggcattctattctataaatgtcactgtagcaatgtggatttttctcttaaaaaacagtgacagctgttgaaatgaagccgcttaaatcttgtcccttttagtttgctatggaagtatgcaaaattattacataaaacctgatgtcatgttctctttatgccatgccatagaacattaatacttttgatttatccttgtacattgagatggctggttaatgtcaatgttggggaaacttttttttccccccttgccggagttgttttttttttttattgtagtgttgaaatgctttgcaaactattcctttgttttcattagacacttttattagcatgagcaccaagcagtttatttgccacagttttcacagtaagcaggaagggtttgataagagctcaaaagcacttgagcactttttcttaggctggagaaaactgagaagcccagttggaactatatagcccatttaaagcaagctccccacttccataagcatatagaagtttgggggataccagaattacactagtcacctcaaatactatttgataggactgtaggtagaaagctattagtattaaagacaaatttaagcaggttttatttttatttattgtgtaatttgacttaaacttagtttttactttctgaggttggtaaattacatgtattgactgttatgaacaaaaagcaaacagttttgggaataattttttttttgttgagttacactgttttaaaggtatcacctatttgatctcatgtctcctcaaaaaaaatagactgggcctgatggctggtaatcttatcactttgggaggctgaggcagcaggatcacttgagcccaggagtttgagaccagcctgggcaacatagtgagaccccatctctacaaagtaaatgtatcgtcaaaatgtttttctgaagtagttttttttataaatatactgtctccttcccaaattgtctcaggctgtctaatactttcactcttaaactctgaccttctgtaatacatttcttaatattcccagtcaggtacaggtaccaactgtatgcagtacagcatgttcactttagggtagaaaacgttactcagtgtgccattgcatagttgatggtctgctctcttaaacaactctttgaaaagaaagtttgttggccgggcgcagtggctcacgcctgtaattccagcactttgggaggccgaggcggatcacttgaggtcaggagttcatgaccagcctggccaacgtggtgaaaccccatctctcctaaaaatacaaaaattagccaggcatggtggcgtgcacctgtaatcccagccactcaggaggctgatgcaggagaatcacttgaacctgggaggcagaggttgcagtgaggcaagatcatgccactgcactccagcctgggcaacagagcgagactttgcctcaaaaaaaaaaaagtttgtgtctattgaatataagaggatccctcttcagtgattgatagcatttttattttttaatttattttgagacagtttcactcttgttgcccaggctggagtgcagtggctcaacttctgtctcccgggttcaagctgttctgcttcagtctcccgagtagctgggattagaggcatgcaccacctggctatttttgtatttttagtagagatggggtttctccatgttggtcaggctggtctcaaactcgcaacctcaggtgatccacccgcctcagcctcctaaagtgctgggattacaggtgtgaatcaccatgcctggcctggtagaattcttataaagaatacttgtagttcatcaaaactgtgacattcaggacctgttctctttattgtctttaagttaaatcctatcttttcttggctttcatcataaaattaggtttccaatgggagtagagggaaaaaaatctgttcttaggttctcttcttatcctgccttttcctagaccacagatttctttaaagccattccttggacctccaggtttcagttaagatttagggcagaggaaccaaaacttctatgctactaaaataaaaatcatgtgcggtcagggacctttttgttctactttgtaggcccggtacctgccacatagtaatcattgaatattccttgaataaattttattctcaatgagtgtgtaacacaaaaaagttctagagcactactatcctaagatttctgcctactctccaagtcccttcctcccaaatttggtatatttcagtgtttacctttgagatgaaggcaattttttaatctggtaaattgtaattgttggtggctgggcatggtggcgcatgtctaatcccaacactttgggaggctgaggcagtgggattgcttgagcccaggagttcaagaccagtctgggcaacacagcaagaccctgtctcaaagaaaagaaaaaaaaatttttttttttttttttttagttgtaagtgctggtgaccgctaacatccttgtgtagatgaagttactaaatttttttttttttttttttttttttttttttttttgagacggagcttcactctcttgcccaggctggagtgcagtagcatgatcttggctcactgcaacctttgctgtccaacttcaagcaattctcctggctcagtctcccaagtagctgggattacaggcgtgcaccaccacacccggctagtttttgtatttttaggagagatggggtttcaccatgttggccaggctggtcttgaactgctgacgtcaggtgatccgcttaccttgacctcccaaagtgttgggattacaggcatgagccactgctcccggcctaaaattttttatattacttggtcgtataaagcattccagtctagtatgacatcactaacaatttcattttgttgataactctgccatgatgtcattagttgttgctgtttgacttttggaagactgataggaaaaatgtacagtattttttccttaagaagtctgtacctaaactttcattaaattttcaaggtccaaatttgtttgagaaaaatattaatattactcaatgtatagcaacaactgcatgaagcgccaaaagagttccagtacatgatctttaagggattattaagttcagaattttgtgaagaaatagaagttaataaacagtcatttgatttgttttgtaattgtcttgtgataacctattttaataaaatttttaaaacatgttattttaataaaattatatgtttaggtaataaactaattagggaagggccttggggttgctaatgaacaaataaaacttgagtaatagatttttctgaaagtttcagtttggtcagctaaaatggattttggtaggttccttatatctatcaattatgtagaagatagctgttctgtggcattcaggacctgttctctttattgtgtgtttaggttttgactcttggatttaatttcaggtcattcctgggagttacagtttagaattatatgcttctatacataaagattacgctagttctgaagtacaggaaaactgtaaaggcaggtgaattaaaattttactttggggtttattattttgagtttttacaggtattttttactctttagtataaaaatacaagtaaaaatttggaataaaccttgacctttaaaagaaatgttatttgttcctttcttgaatgaataacaaatggtattagcatagatacggttttattttctgcattttacttattctagcaaacattttaagtgttattagatttttaaatttctcgaaagttatacatagtcttacactatgcatcttccagtatttagctttttgttaaatcatgtaatagaaaggtgattactgctaattaaacattgggaatttatgcacctaatggtggtgttaaaagatacccatagcagagaatgtaatataaacaaatacctcaaagtcctttaattttcttgtaacctaaattaggtgaaaggtgcaatgtgtctgaactccaatatatgtatttctagatatttctacattctgtttaaaaacagtaaaattgaaatgtctttatcaattgtgctatttgtaggtggagactccctgatctatttttgtcattaggttgatctaggttagcactgtatactatcttcataaaatcaattagtgtggtatgaaccttctgattggtattagatgagttcctctataaaccagtaatatttaaataagaaagaatgcagttaggaggcaattgtaatagccctggcaaaggacgatggagccttgaaccaaaatactggttgtagagatggaggaaaaatcaggcagtatttaaatgatagaattcgagacctgttgacagatttcagactgaaagagttaaaagtggctcttgggcttttgctagtacctttagggttgcctgggagtatagaattcattttcatatgttttgcttgtcatcagccaggggagctatatcctgtagacagccagaaataaagacatttattgagcgagatgggtagactaaagatatcttcgttgtaagtgggtatagatgaagtggccaaggagtggaaaaaaaggataaaattggtcacatctagacataagagacaggagtaagagcctttggcagtatatggtaggaggaaaatcaaagtactgttacgaaggccaagaaaaattttgagagtttttccatgcagttttggatgctgcaaaaaaatgagatagtctttatcttgacatttattaagtatgtatttgttggacatagttctaagtgtttgacacatactaatttttttatggggggtgaccaggtgaataccccttgtgggcatggtatactgtgtcaccccacttactgggcacatttatgtcatttcacagaaatgaggaagctgaggcagaaaaggtttagtagcttgtccatattgcattgccagaagaagaaacagagctaggaaattctaacccagtagtcaagttacaaagtctcattttagtttctatgccatatggcttcacattgaagcatgcttgatggattgggtgactgactagtagtcattggtaaactcagcattttcaggtgatgagttggagctggatgtcattttaaaatagtggattgtttggagagaggaaattggtatgagtagtagtgccttccaaaatttggggagggataagggcaagcatttaaaatataactaaggtttcaatttagttttaggctaagcgatgtgaagatatttatgtggtaatgggcaaattagtggaagaatagttgagtccagggaagaggtaatacggaatgaaactggaaggtgtacgcgaattggagttagggataagcaggcagggaataaattggccttggaccgtaaagaaggtacaccatttcttacacatgtgtcacataaattttcaaatgtatggctatgttgggaaagcttaatggcccaatgaacttggaaactttttgtattcatttgctgatagggtctaatattttctgggaaatgacttacttggaaaatactagctttattatttactgattggtataactttgcagtatcaaagttagtctgttttagtttctttctttctttttttttttttgagacaagtctcactctgttgcccaagctggagtgcagtggtgtgatctcggctcactgcaacctccgcctctcgggttcaagcagttctgctgctgcagcctccccagtagctgggactacaggcgcacgccgccacacccagcttgtgtgtgtgtttgtgttttaatagagacgggggactacaggcccacgctgccacacccagcgtgtgtgtgtgtgtgtgtgtgtgtgtgtgtgtgtgtgtgttttagtagagacgggggactacaggcacacgccgccacacccagcttgtgtgtgtgtgtgttttagtagagacggggtttcttttctttttcttctttttttttttttttgagacggagtctcgctctgtcgcccaggctggagtgcagtggcgcaatatcagctcactgcaagctctgcctcccaggttcacgccattctcctgcctcagcctcccgagtagctgggactataggcgcccgccaccacgcccggctaatttttttgtatttttagtagagatggggtttcaccgtgttagccaggatggtctcgatctcctgacctcatgatccacccgcctcagcctcccaaagtgctgggattacaggcttgagccaccgcgcccggcctgagacggggtttcaccctgttgttcaggctggtctggaactcaccctgagctcaggcagtctgcccaccttggcctcccaaagtgctaggattacaggtgtgagccactgcacctggcttgttttagtttatctgtaaatggtgaatgaagccaggtagtctggagtgttgcaccagcaggaggtttccatgtaatctagtgatgtattagaaggaacatatagccgggcacagtggctcatgccctgtaatcccagcactttgggaggcagagacaggcggatcacctgaggttgggagttcgaggccagcctgaccaacgtggagaaaccccatctctactaaaaatagaaaattagctgggcgtggtggtgcatgcctgtaattccagctactcgggaggctgaggcaggagaattgcttgatcctgggaggaggaggttgcggtgggctgagattgcaccattgcactccagcctggacaacaagagcgaaagtccatctcaaaaaaaaaaacaacagcaggaaggaacatactatcacaacaagatgttgaggaataatcagtttcactatataaggttggggttttaatattccaaagaaagctcaaaatgatctttgttctcagtgacatgcatttagctaaaactggacatttatatcttgatcagcccattgttatagactctttatatagtcccttctcctgccttactagaaagggaaagtagcctgttttaatttagtaggtgattgatttagacatagtggctaactctaaacacagtatacagaaacagtttaattactctgtagaaatacgtatttgggtaccagtagtcttatttttgttttgtgagtgtaggttaggtctgtaattttgaattatgttccacagagcagcttcagtgacagaggagccagtcatttggggatttggttcttttcctctgtaaacctaggataattttacttaggtcagcatgaaagtacagtggtatgattggtcaaagatatatttgaaatattatcataaggtatcataaagattggttaatctttaggagtcaaagtcacatttcaattgctacctccattggtatttttccgttaaaagtttttgggtttttctgagacgtggggtcttacagtttggccaggctgaagtgcagtggctgttcactggcacgatcccaccactgagtaggctttaagagttaatacgtttcatttaggttacattttattattaatctgtgtatttggattgtggtctttctttcaaacagaattcaaagaagctttttcactatttgacaaagatggtgatggaactataacaacaaaggaattgggaactgtaatgagatctcttgggcagaatcccacagaagcagagttacaggacatgattaatgaagtagatgctgatggtaagtcttcaattttgtggggctgggaggggttgaagaagtgatacttagatgtttccactaaacctttgctgtttgcttatatgtttccactaaagctttgatgtttccactaaaccatttcaggtaatggcacaattgacttccctgaatttctgacaatgatggcaagaaaaatgaaagacacagacagtgaagaagaaattagagaagcattccgtgtgtttgataaggtacgtcaaggactggatatgttaaattttgaggatgaaatgaagataccaggactcattatgaagacttgtgtttttttggttgtttttttttttttttttttttttttttttgatgatttaccaacatattttaattaccaagcaaaagctttttaagaattcagtatagactttctaatatatgtattgcgttcatcttgtcaaaggaggtgtcacttgactttgggactaggaaataatgatttcaatgtaggacattttgcttggctcttaatgacatttgtaggtcaactgtgtagatttgtatgcatttctaaagtatgtttttcccccaatgtgaaatttagtagtaaacttaataaatttccattccaactctcaagtctgtaatttgactcagaaactatactaaattttttgctaggatggcaatggctatattagtgctgcagaacttcgccatgtgatgacaaaccttggagagaagttaacagatgaagaagttgatgaaatgatcagggaagcagatattgatggtgatggtcaagtaaactatgaaggtaaatgtttcagtctcacgcctcattcttcactttgatttttaagataagaggctctttgttagggaactgatcgaaattagtgacccttcccctgaaattaggttgctaaaacagttacttacatttaaccttcttaaaattcagagtgttgtctgcagactaggtaacattgctctgacttgagaacttaatttagaaatatttactatcaggttctatccctacacctggaatcagcattttaataggattcttgggtgattcatgtataaagtttgagaagcactgttcagtgtttgtgtgattgtggaacaatgtggaaagcaaacttattccaagtttcctaaaatgaaattaatgtgactttctttccccgcactgtattgtcttttttctttaattggctttagtctgaaactgaagtttacatgtgcttcaaaagtatcgtatctactaacttttaagatggccatatcaggaagcaaggcatatgaaactgaaggattttgagtaaaactctgtatttttttcatgatgtaactacttaacttagaaaagagcataaaatgtaatgttataaaaattaaacctagcccatagcattgaatttacaatattgtcttgtaatccagcagacttaaaattcaagtctaaactaagagccaagaatgctcttttttatattggcctatctaaagcgttaatttggctcttactaataaacctgaatagttatggttaatgaagttccagcctgggcaataaactagcttccctctgtacttaatggtaattctgaggaaagagaggaatggaaagagtactcagtaattgagtaaatgtgattttttttttttttttttttttttggtcttttgctattgactcattttttgtgtacttcttctttttcagagtttgtacaaatgatgacagcaaagtgaagaccttgtacagaatgtgttaaatttcttgtacaaaattgtttatttgccttttctttgtttgtaacttatctgtaaaaggtttctccctactgtcaaaaaaatatgcatgtatagtaattaggacttcattcctccatgttttcttcccttatcttactgtcattgtcctaaaaccttattttagaaaattgatcaagtaacatgttgcatgtggcttactctggatatatctaagcccttctgcacatctaaacttagatggagttggtcaaatgagggaacatctgggttatgccttttttaaagtagttttctttaggaactgtcagcatgttgttgttgaagtgtggagttgtaactctgcgtggactatggacagtcaacaatatgtacttaaaagttgcactattgcaaaacgggtgtattatccaggtactcgtacactatttttttgtactgctggtcctgtaccagaaacattttcttttattgttacttgctttttaaactttgtttagccacttaaaatctgcttatggcacaatttgcctcaaaatccattccaagttgtatatttgttttccaataaaaaaattacaatttacccaatggttgctctgcatctgagtcatttaactgttgaagtctaataattttgaaaataaaatatggcattggtttctgcttggta

SEQ ID NO: 3 - DNA, 16 bp, Artificial Sequence
  Synthetic oligonucleotide
ggtcttcactttgctg

SEQ ID NO: 4 - DNA, 16 bp, Artificial Sequence
  Synthetic oligonucleotide
cccagatgttccctca

SEQ ID NO: 5 - DNA, 16 bp, Artificial Sequence
  Synthetic oligonucleotide
aagcgctaccggtttc

SEQ ID NO: 6 - DNA, 16 bp, Artificial Sequence
  Synthetic oligonucleotide
gtgtacgagtacctgg

SEQ ID NO: 7 - DNA, 16 bp, Artificial Sequence
  Synthetic oligonucleotide
ggactaattcgcctcc

SEQ ID NO: 8 - DNA, 16 bp, Artificial Sequence
  Synthetic oligonucleotide
gtccatagtccacgca

SEQ ID NO: 9 - DNA, 16 bp, Artificial Sequence
  Synthetic oligonucleotide
gcagattttaagtggc

SEQ ID NO: 10 - DNA, 16 bp, Artificial Sequence
  Synthetic oligonucleotide
agtcagttggtcagcc

SEQ ID NO: 11 - DNA, 16 bp, Artificial Sequence
  Synthetic oligonucleotide
gggaagtcaattgtgc

SEQ ID NO: 12 - DNA, 16 bp, Artificial Sequence
  Synthetic oligonucleotide
tttgacagtagggaga

SEQ ID NO: 13 - DNA, 16 bp, Artificial Sequence
  Synthetic oligonucleotide
gcagagcaaccattgg

SEQ ID NO: 14 - DNA, 16 bp, Artificial Sequence
  Synthetic oligonucleotide
tcatgtcctgtaactc

SEQ ID NO: 15 - DNA, 16 bp, Artificial Sequence
  Synthetic oligonucleotide
gcagaagggcttagat

SEQ ID NO: 16 - DNA, 16 bp, Artificial Sequence
  Synthetic oligonucleotide
gtggctaaacaaagtt

SEQ ID NO: 17 - DNA, 16 bp, Artificial Sequence
  Synthetic oligonucleotide
gcttctttgaattctg

SEQ ID NO: 18 - DNA, 16 bp, Artificial Sequence
  Synthetic oligonucleotide
tctgcagcactaatat

SEQ ID NO: 19 - DNA, 16 bp, Artificial Sequence
  Synthetic oligonucleotide
tgccatcattgtcaga

SEQ ID NO: 20 - DNA, 16 bp, Artificial Sequence
  Synthetic oligonucleotide
gtacaggaccagcagt

SEQ ID NO: 21 - DNA, 16 bp, Artificial Sequence
  Synthetic oligonucleotide
cctcatttgaccaact

SEQ ID NO: 22 - DNA, 16 bp, Artificial Sequence
  Synthetic oligonucleotide
tccctcatttgaccaa

SEQ ID NO: 23 - DNA, 16 bp, Artificial Sequence
  Synthetic oligonucleotide
gttccctcatttgacc

SEQ ID NO: 24 - DNA, 16 bp, Artificial Sequence
  Synthetic oligonucleotide
ccagatgttccctcat

SEQ ID NO: 25 - DNA, 16 bp, Artificial Sequence
  Synthetic oligonucleotide
acccagatgttccctc

SEQ ID NO: 26 - DNA, 16 bp, Artificial Sequence
  Synthetic oligonucleotide
aacccagatgttccct

SEQ ID NO: 27 - DNA, 16 bp, Artificial Sequence
  Synthetic oligonucleotide
taacccagatgttccc

SEQ ID NO: 28 - DNA, 16 bp, Artificial Sequence
  Synthetic oligonucleotide
aggcataacccagatg

SEQ ID NO: 29 - DNA, 16 bp, Artificial Sequence
  Synthetic oligonucleotide
aaaggcataacccaga

SEQ ID NO: 30 - DNA, 16 bp, Artificial Sequence
  Synthetic oligonucleotide
aaaaaggcataaccca

SEQ ID NO: 31 - DNA, 16 bp, Artificial Sequence
  Synthetic oligonucleotide
actcaccatgctgcaa

SEQ ID NO: 32 - DNA, 16 bp, Artificial Sequence
  Synthetic oligonucleotide
aagatgtcaccttgcc

SEQ ID NO: 33 - DNA, 16 bp, Artificial Sequence
  Synthetic oligonucleotide
ggaggtttcagttggc

SEQ ID NO: 34 - DNA, 16 bp, Artificial Sequence
  Synthetic oligonucleotide
agtgccattttcttag

SEQ ID NO: 35 - DNA, 16 bp, Artificial Sequence
  Synthetic oligonucleotide
cagtcagttggtcagc

SEQ ID NO: 36 - DNA, 16 bp, Artificial Sequence
  Synthetic oligonucleotide
gctcttcagtcagttg

SEQ ID NO: 37 - DNA, 16 bp, Artificial Sequence
  Synthetic oligonucleotide
acctgcaatctgctct

SEQ ID NO: 38 - DNA, 16 bp, Artificial Sequence
  Synthetic oligonucleotide
ttgtgccattacctga

SEQ ID NO: 39 - DNA, 16 bp, Artificial Sequence
  Synthetic oligonucleotide
gtcagaaattcaggga

SEQ ID NO: 40 - DNA, 16 bp, Artificial Sequence
  Synthetic oligonucleotide
ccatcattgtcagaaa

SEQ ID NO: 41 - DNA, 16 bp, Artificial Sequence
  Synthetic oligonucleotide
tcttgccatcattgtc

SEQ ID NO: 42 - DNA, 16 bp, Artificial Sequence
  Synthetic oligonucleotide
actgtctgtgtctttc

SEQ ID NO: 43 - DNA, 16 bp, Artificial Sequence
  Synthetic oligonucleotide
tcttcttcactgtctg

SEQ ID NO: 44 - DNA, 16 bp, Artificial Sequence
  Synthetic oligonucleotide
tagccattgccatcct

SEQ ID NO: 45 - DNA, 16 bp, Artificial Sequence
  Synthetic oligonucleotide
gcactaatatagccat

SEQ ID NO: 46 - DNA, 16 bp, Artificial Sequence
  Synthetic oligonucleotide
ccaaggtttgtcatca

SEQ ID NO: 47 - DNA, 16 bp, Artificial Sequence
  Synthetic oligonucleotide
tcttcatctgttaact

SEQ ID NO: 48 - DNA, 16 bp, Artificial Sequence
  Synthetic oligonucleotide
tgtcatcatttgtaca

SEQ ID NO: 49 - DNA, 16 bp, Artificial Sequence
  Synthetic oligonucleotide
aacacattctgtacaa

SEQ ID NO: 50 - DNA, 16 bp, Artificial Sequence
  Synthetic oligonucleotide
tacagataagttacaa

SEQ ID NO: 51 - DNA, 16 bp, Artificial Sequence
  Synthetic oligonucleotide
ttttttgacagtaggg

SEQ ID NO: 52 - DNA, 16 bp, Artificial Sequence
  Synthetic oligonucleotide
tactatacatgcatat

SEQ ID NO: 53 - DNA, 16 bp, Artificial Sequence
  Synthetic oligonucleotide
tggaggaatgaagtcc

SEQ ID NO: 54 - DNA, 16 bp, Artificial Sequence
  Synthetic oligonucleotide
gggaagaaaacatgga

SEQ ID NO: 55 - DNA, 16 bp, Artificial Sequence
  Synthetic oligonucleotide
gtaagataagggaaga

SEQ ID NO: 56 - DNA, 16 bp, Artificial Sequence
  Synthetic oligonucleotide
gacagtaagataaggg

SEQ ID NO: 57 - DNA, 16 bp, Artificial Sequence
  Synthetic oligonucleotide
ggacaatgacagtaag

SEQ ID NO: 58 - DNA, 16 bp, Artificial Sequence
  Synthetic oligonucleotide
catgcaacatgttact

SEQ ID NO: 59 - DNA, 16 bp, Artificial Sequence
  Synthetic oligonucleotide
agccacatgcaacatg

SEQ ID NO: 60 - DNA, 16 bp, Artificial Sequence
  Synthetic oligonucleotide
ccagagtaagccacat

SEQ ID NO: 61 - DNA, 16 bp, Artificial Sequence
  Synthetic oligonucleotide
agtttagatgtgcaga

SEQ ID NO: 62 - DNA, 16 bp, Artificial Sequence
  Synthetic oligonucleotide
caactccatctaagtt

SEQ ID NO: 63 - DNA, 16 bp, Artificial Sequence
  Synthetic oligonucleotide
catgctgacagttcct

SEQ ID NO: 64 - DNA, 16 bp, Artificial Sequence
  Synthetic oligonucleotide
acaacatgctgacagt

SEQ ID NO: 65 - DNA, 16 bp, Artificial Sequence
  Synthetic oligonucleotide
tattgttgactgtcca

SEQ ID NO: 66 - DNA, 16 bp, Artificial Sequence
  Synthetic oligonucleotide
cgttttgcaatagtgc

SEQ ID NO: 67 - DNA, 16 bp, Artificial Sequence
  Synthetic oligonucleotide
ccagcagtacaaaaaa

SEQ ID NO: 68 - DNA, 16 bp, Artificial Sequence
  Synthetic oligonucleotide
ggctaaacaaagttta

SEQ ID NO: 69 - DNA, 16 bp, Artificial Sequence
  Synthetic oligonucleotide
aagtggctaaacaaag

SEQ ID NO: 70 - DNA, 16 bp, Artificial Sequence
  Synthetic oligonucleotide
tttaagtggctaaaca

SEQ ID NO: 71 - DNA, 16 bp, Artificial Sequence
  Synthetic oligonucleotide
caacttggaatggatt

SEQ ID NO: 72 - DNA, 16 bp, Artificial Sequence
  Synthetic oligonucleotide
ctcataaacacctccc

SEQ ID NO: 73 - DNA, 16 bp, Artificial Sequence
  Synthetic oligonucleotide
cccagcgcctcataaa